European Patent Application EP 4 722 355 A1, published April 8, 2026. Title: Verfahren zur Herstellung von 2,5-Furandicarbonsäure. Applicant: Annikki GmbH. Application EP. The sequence listing filed with the application follows.

SEQUENCE LISTING (18 sequences)

SEQ ID NO: 1 - DNA, 1410 bp, Pseudomonas nitroreducens
  source 1..1410: mol_type = genomic DNA
atgtcacgctatgaactgctgatcgatggtcgcctgcaggcggccgagcactacgaccgggtgatcgacccggccagcgaagaaatcgttggcgaagccgcccgcgccagcctggagcaggtcgacgcggcggtggatgccgcacaccgcgccttcccggcctgggccaccgatctcgacgtccgccgccagagcctggcccgagccgccgaacgagtacgcgagaatgcccaggcgctggccgagctgatcacccgcgaacagggtcgcccactgcgctcgaccctggaggaagtggctggcgtcgccgccactttcgagcaccacgcgcagctggagctacccgccgacacccagttgcgcgacgacggcgagcgcctggtgcgcatcacccgcaaaccgctgggggtggtcgccgcgatcaccccgtggaacgtcccgctgatcctgctggtattgaagatcgcgcctgccctgcacgccggcaacaccgtggtggccaagccctcggagcacacgccgctgtctaccctgctgctggcgcgactgctgggcgatgtgttccccgctggcgtgttcaacgtggttgccggtgcgggcgaggttggcgaacacctggtacgtcatccgcgggtgcgccacgtgaccttcaccggcagcgtcgccaccggcaagcgcctgtatgccggcgcgggggacgacctcaagcgtcttaccctggaactgggcggcaacgacgccgcgctggtactggaagacgccgacctcgacgccatcgtcgaaccgctgttctggggcgccttctggaacagcggccaggtgtgctttgcgatcaagcgcctgtacgtgcatgacagcctgttcgaaccgttactggcgaaactcgccgagcgcgcccagcgcacccgcctcggtcatgggctcgacccgcagacggaactggggccgctgaccaacgcacagcaactggaacgggtcatcgccctggtggaagacgccaaggctcacggagcacgcatccgcagcggcggcgtacggcccgacggtcccggctacttctacccgccgaccctggtcagcggcgtggcggccggcgtcgcgctggtggacgaggaacagttcggcccggtgttgccggtgatctccttccgcaacgaagaggacgccattacccaggccaacgccagccactacggcctcggcgcctcggtgtggacccgcgacctggcgcgcggcgaagccatcgccaggcggctggaggcgggcctggcctgggtcaaccagcacggccacatccagcccggcgcgcccaagggcgggcacaagtggagcgggctcggctacgaaggcgggcagcgcggctatgaggccttcagcgagctgcaggtgctgaacatttcgcggcgctaa

SEQ ID NO: 2 - protein, 469 aa, Pseudomonas nitroreducens
MSRYELLIDGRLQAAEHYDRVIDPASEEIVGEAARASLEQVDAAVDAAHRAFPAWATDLDVRRQSLARAAERVRENAQALAELITREQGRPLRSTLEEVAGVAATFEHHAQLELPADTQLRDDGERLVRITRKPLGVVAAITPWNVPLILLVLKIAPALHAGNTVVAKPSEHTPLSTLLLARLLGDVFPAGVFNVVAGAGEVGEHLVRHPRVRHVTFTGSVATGKRLYAGAGDDLKRLTLELGGNDAALVLEDADLDAIVEPLFWGAFWNSGQVCFAIKRLYVHDSLFEPLLAKLAERAQRTRLGHGLDPQTELGPLTNAQQLERVIALVEDAKAHGARIRSGGVRPDGPGYFYPPTLVSGVAAGVALVDEEQFGPVLPVISFRNEEDAITQANASHYGLGASVWTRDLARGEAIARRLEAGLAWVNQHGHIQPGAPKGGHKWSGLGYEGGQRGYEAFSELQVLNISRR

SEQ ID NO: 3 - DNA, 1410 bp, Methylovorus glucosotrophus
  source 1..1410: mol_type = genomic DNA
atgtcgacatttcatttacttattgatggccatctgcaagccagtgaccaatccgatgtggtgatcaaccccgcgaccgagctggaagtcgggcgtgccccacgtgccagcgccacccaggtcgaccaggcagtggaagccgcacatcaggcatttcatcgctgggcatcacagcctgaggtgcgccagcaggcactgctgggcgcggccgccgccattcgccagcatgccgatgccctggcacgcctgatcacgcaagagcaggggcggccattgcactttacccagggcgaggtggccggggctgctgctacctttgaacactatgccgggtttgccgcgccatcggatgtggtgctgcagcaggacgaacaaaagcgggtcagcattgagcgcaggccgtttggcgtagtggctgccattacgccctggaatgtgcccatcatcctgctggtactgaaaatcgccccggccttgaaggctggcaataccgtggtcgccaagccatcggaatacaccccgctttctaccttgtacctgggtgaaattctgaaagatgtatttccgcccggcgtgctgaacgtgatagccggtgacggtcaggtgggggcgcgcctggcatcgcatccgctggtgcagaaggtgacgttcaccggcagcgtggcaaccggaaaaaaactctatgccagcgccgcgcaggatgtaaaacgcctgacgctggaactgggcggtaacgatgcggccatcgtgctggacgatgccaatgtcgatgccattgccgagaagattttctggggcgccttctggaatagcggtcaggtgtgctttgccatcaagcgcctctatgtgcacgagcgtgttttccagcccttgctcgatgccctggtgaaacgcgcgcaaaaaacccgcgtgggcgatggccagctgccgggtaccgagctggggccgcttaccaacaaagcccagtttgagcgcgtgatatcgctggtggaagacgccagacgccatggcgccaccattcattcaggcggtgctgcattgcctggccccggctatttctatccgcccaccctggtcaccggcataggcgcaggtgtcgcgctggtggatgaagagcagttcggaccagtattgccgctgattcctttccgtgatgagcaagaggcggtgcgtcaggccaacgacagtccgtttggtctgggcgcttcggtttggaccgccaatcccgaacgcggcctggcgctggtacgccagctccaggccgggctcgcctgggtcaaccagcatggcgatatccatcccggtgcgcccaagggcggctacaaatccagtggccttggctacgagggcgggctgcgtggctatgacgagttcagcgagctgcaagtcgtcaatgcggcgctggtttaa

SEQ ID NO: 4 - protein, 469 aa, Methylovorus glucosotrophus
MSTFHLLIDGHLQASDQSDVVINPATELEVGRAPRASATQVDQAVEAAHQAFHRWASQPEVRQQALLGAAAAIRQHADALARLITQEQGRPLHFTQGEVAGAAATFEHYAGFAAPSDVVLQQDEQKRVSIERRPFGVVAAITPWNVPIILLVLKIAPALKAGNTVVAKPSEYTPLSTLYLGEILKDVFPPGVLNVIAGDGQVGARLASHPLVQKVTFTGSVATGKKLYASAAQDVKRLTLELGGNDAAIVLDDANVDAIAEKIFWGAFWNSGQVCFAIKRLYVHERVFQPLLDALVKRAQKTRVGDGQLPGTELGPLTNKAQFERVISLVEDARRHGATIHSGGAALPGPGYFYPPTLVTGIGAGVALVDEEQFGPVLPLIPFRDEQEAVRQANDSPFGLGASVWTANPERGLALVRQLQAGLAWVNQHGDIHPGAPKGGYKSSGLGYEGGLRGYDEFSELQVVNAALV

SEQ ID NO: 5 - DNA, 1410 bp, Pseudomonas multiresinivorans
  source 1..1410: mol_type = genomic DNA
atgtcgcgctatgaactgctgatcgatggtcgcctccaggcggccgagcactacgaccgggttatagacccggccagcgaagaactcgtcggcgaagccgcccgcgccagcctggagcaggtcgacgcggcggtggacgccgcgcaccgcgccttcccaacctgggccaccgatctcgacggccgccgccagagcctggcccgagccgccgaacgagtacgcgagaacgcccaggcgctggccgagctgatcacccgcgaacagggtcgcccgctgcgctcgacactggaggaagtggcgggcgtcgccgccactttcgagcaccacgcacatctggagcttcccgccgatacccagttgcgcgacgacggcgaacgcctggtgcgcatcacccgcaaacccctgggggtggtcgccgcaatcaccccgtggaacgtcccgctgatcctgctggtgctgaagatcgcgcccgccctgcatgccggcaacaccgtggtggccaagccctcggaacacacgccgctgtccaccctgctgctggcgcgactgctgggcgatgtgttccctgctggcgtgttcaacgtgattgccggtgcaggcgaggtcggcgaacacctggtgcgccatccccgagtgcgccacgtgaccttcaccggcagcgtcgccaccggcaagcgcctgtatgccggcgcagcggacgacctcaagcgcctgaccctggaactgggcggcaacgatgccgcgctggtgctggaagatgccgacctcgaagccatcgtcgaaccgctgttctggggcgccttctggaacagcggccaggtgtgcttcgcgatcaagcgcctgtacgtgcatgaaagcctgttcgaaccgctgctggccaaactcgccgaacgcgccgagcgcacccgcctcggccatgggctcgacccgcagacggaactggggccgctgaccaacgcgcagcaactggaacgggtcatcaccctggtggaagacgccaaggctcacggagcgcgcatccacagcggtggcacgcggcccgacggccccggttacttctacccgccgaccctggtcagcggcgtggcggccggtgtcgcgctggtggatgaggaacagttcggcccggtgctgccggtgatcccgttccgcgacgaagaggacgccatcgcccaggccaacgccagcccctacggcctcggcgcctcggtgtggacccgcgacctggcgcgcggcgaagccatcgccgaacggttggaggcgggcctggcctgggtcaaccagcacggccacatccagcccggcgcgcccaagggcgggcacaagtggagcgggctcggctacgaaggcgggcaacgcggttacgaggccttcagcgagctgcaggtgctcaacatttcgcggcgctga

SEQ ID NO: 6 - protein, 469 aa, Pseudomonas multiresinivorans
MSRYELLIDGRLQAAEHYDRVIDPASEELVGEAARASLEQVDAAVDAAHRAFPTWATDLDGRRQSLARAAERVRENAQALAELITREQGRPLRSTLEEVAGVAATFEHHAHLELPADTQLRDDGERLVRITRKPLGVVAAITPWNVPLILLVLKIAPALHAGNTVVAKPSEHTPLSTLLLARLLGDVFPAGVFNVIAGAGEVGEHLVRHPRVRHVTFTGSVATGKRLYAGAADDLKRLTLELGGNDAALVLEDADLEAIVEPLFWGAFWNSGQVCFAIKRLYVHESLFEPLLAKLAERAERTRLGHGLDPQTELGPLTNAQQLERVITLVEDAKAHGARIHSGGTRPDGPGYFYPPTLVSGVAAGVALVDEEQFGPVLPVIPFRDEEDAIAQANASPYGLGASVWTRDLARGEAIAERLEAGLAWVNQHGHIQPGAPKGGHKWSGLGYEGGQRGYEAFSELQVLNISRR

SEQ ID NO: 7 - DNA, 1521 bp, Raoultella ornithinolytica
  source 1..1521: mol_type = genomic DNA
atgcgttatgcacatcctggcaccccgggcgccttagtttcattcaagtccgcatacggtaactatattgacggtcaatttgtcgaaccgctcggcggcgaatactttatgaatacctcccccgtggacgggagtgacattgcacaatttccccgctccgatgccaaagatatcgattttgctcttgatgccgcacaccgcgccgcggaagcctgggggaaaacatcggtacagcatcgttccaacctgctgcttcaggtcgccgatcggattcaggagaacctggaatatctggcgattgctgaaagctgggacaatggtaaaccggtgcgcgaaacgctgaatgccgatctgccgttggcggtcgatcacttccgctattttgccggctgtctgcgggcacaggaggggagtactgcggaaattgatgaaaccaccgtggcctatcacttccatgaaccgctgggcgtagtcgggcaaattattccgtggaactttccgctgctgatggcggcctggaagctggcgccggcgctggcggccgggaactgtgtggtgctcaagccggcagagcagacgccgctgagcatcacgctgctgctggaaattattggcgacctcttcccgccgggcgtcctgaacgtggtgcagggcttcggtaaagaggccggtgaagcgctggcaaccagcaagcgtattgccaaaattgcctttaccggctcaacgcccgtcggacggcatattctggcctgcgcggcggagaacattattcccgccaccgttgagctgggcggcaagtcgccaaatatctattttgccgatgtgatggacggagaagaagagtttatcgagaaggcggtggaggggctggtgctgggcttcttcaaccagggcgaagtatgtacctgcccatcgcgcgccctgatccatgaatccatctacgagccgtttatggagcgagtgatggcgaaggtggcccagattcgccgcggcgatccctttgataccgacaccatgatcggggcacaggcatcacgccagcagttcgataagatcctgtcgtacattaagattgcccgcgaagagggggggcagatcctgaccggcggagaacgcgccagtattacggctgaactggataatggttactacattcagccaactctgattaaggggcgcaatgatatgcgcagcttccaggaagagatttttggcccggtcatcggcgtcacgaccttcaaagatgaggcagaagcgctggaaatagccaaccagactcagtttgggctcggcgccggcgtctggacccgcgacagcaatctggcgtaccgaatggggcgtgggattaaagccggtcgtgtctggaccaactgttatcacgtctacccggcccatgccgcgtttggcggctataaacagtcaggcgtcggtcgtgaaactcataaaatggcccttgatgcctatcaacagacgaaaaacctgctggtgagctacggtaccgcgccgttaggactgttttaa

SEQ ID NO: 8 - protein, 506 aa, Raoultella ornithinolytica
MRYAHPGTPGALVSFKSAYGNYIDGQFVEPLGGEYFMNTSPVDGSDIAQFPRSDAKDIDFALDAAHRAAEAWGKTSVQHRSNLLLQVADRIQENLEYLAIAESWDNGKPVRETLNADLPLAVDHFRYFAGCLRAQEGSTAEIDETTVAYHFHEPLGVVGQIIPWNFPLLMAAWKLAPALAAGNCVVLKPAEQTPLSITLLLEIIGDLFPPGVLNVVQGFGKEAGEALATSKRIAKIAFTGSTPVGRHILACAAENIIPATVELGGKSPNIYFADVMDGEEEFIEKAVEGLVLGFFNQGEVCTCPSRALIHESIYEPFMERVMAKVAQIRRGDPFDTDTMIGAQASRQQFDKILSYIKIAREEGGQILTGGERASITAELDNGYYIQPTLIKGRNDMRSFQEEIFGPVIGVTTFKDEAEALEIANQTQFGLGAGVWTRDSNLAYRMGRGIKAGRVWTNCYHVYPAHAAFGGYKQSGVGRETHKMALDAYQQTKNLLVSYGTAPLGLF

SEQ ID NO: 9 - DNA, 1452 bp, Comamonas testosteroni
  source 1..1452: mol_type = genomic DNA
atgatcgaacaaaaaatgctgatcgccggccaggaatgtgcagccggcaatggcgcaacgtttgagcgcaagaatccgctggatggatccgtcgccacacgcgccccggcagccacgaccgaggatgcgattcgcgcctgcgacgctgctgcagccgccttccccgcctggtcgcaactggggccgaacgcccgccgcgccatgctgatgaaggcctcgcaggcactggaagccaagggcgaagcgattgctgcggccatggctgccgagaccggcgcctcgggcatctgggccggcttcaacgtgcatctggccgccagcatgctgctggaggcggcttcgctgaccacgcagatcaatggcgagatcattccctccgacgtacccggcagcgtggccatggccgtgcgccagcccgccggcgtggtactcggtatcgcgccctggaatgctcccgtgatcctggccgtgcgcagcatctccacggccctggcctgcggcaacaccgtgattctcaagggctcggaactctgccccgccacccacggcctgatcatcgaggcactgcaggacgcaggcctgcccgccggcgtggtgaactttgtgaccaatgcgcccgccgatgcgggcagcgtggtcgaagccatcgtggcccacccggccgtgcgccgcgtgagctttaccggctccaccaaggtgggccgcatcatcggccagacctgcgccaggcacttgaagcctgcgctgctggagcttggcggcaaggcccccttcctggtgctcgacgatgccgatatcgatgcggccgtgaacgccgccacctttggcgcgtttgccaactcgggccagatctgcatgtctaccgagcgctttgtggtggataacaaggtggccgacgagttcatcgccaagtttgccgccaaggccagcagcctgccgctgggcgacccgcgcaagggccccgtggtgctgggctcggtcgtcgatctggctacggtggagcgctgcaatgccatgatcgacgacgcgctggccaagggcgcaaaaatcgtctgcggcggcaaggccgagagcacgctgatgcccgccacgctgatcgaccatgtgacgccggcgatgcgcatattccacgaggagacctttggcccggtcaaaggcatcgtgcgcgtgaacggcgaggaagaagccattgccacggccaatgacaacgagttcggtctgtcctccgcagtcttcacccgggacacggcccgcggctggcgtgtggcggcacgcatcgaggccggcatctgccacatcaacggccccacggtgcatgacgaagcccagatgccgtttggtggcgtcaaggcctcgggctatggccatttcgggggccagcagggcatcaatgcctttaccgaaacccgctgggtgaccatgcagaccgcagaacgccactatccgttctaa

SEQ ID NO: 10 - protein, 483 aa, Comamonas testosteroni
MIEQKMLIAGQECAAGNGATFERKNPLDGSVATRAPAATTEDAIRACDAAAAAFPAWSQLGPNARRAMLMKASQALEAKGEAIAAAMAAETGASGIWAGFNVHLAASMLLEAASLTTQINGEIIPSDVPGSVAMAVRQPAGVVLGIAPWNAPVILAVRSISTALACGNTVILKGSELCPATHGLIIEALQDAGLPAGVVNFVTNAPADAGSVVEAIVAHPAVRRVSFTGSTKVGRIIGQTCARHLKPALLELGGKAPFLVLDDADIDAAVNAATFGAFANSGQICMSTERFVVDNKVADEFIAKFAAKASSLPLGDPRKGPVVLGSVVDLATVERCNAMIDDALAKGAKIVCGGKAESTLMPATLIDHVTPAMRIFHEETFGPVKGIVRVNGEEEAIATANDNEFGLSSAVFTRDTARGWRVAARIEAGICHINGPTVHDEAQMPFGGVKASGYGHFGGQQGINAFTETRWVTMQTAERHYPF

SEQ ID NO: 11 - DNA, 1521 bp, Corynebacterium glutamicum
  source 1..1521: mol_type = genomic DNA
atgactgtctacgcaaatccaggaaccgaaggctcgatcgttaactatgaaaagcgctacgagaactacattggtggcaagtgggttccaccggtagagggccagtaccttgagaacatttcacctgtcactggtgaagttttctgtgaggtcgcacgtggcaccgcagcggacgtggagcttgcactggatgctgcacatgcagccgctgatgcgtggggcaagacttctgtcgctgaacgtgctctgatcctgcaccgcattgcggaccgcatggaagagcacctggaagaaatcgcagttgcagaaacctgggagaacggcaaggcagtccgtgagactcttgctgcagatatcccactggcaatcgaccacttccgctactttgctggcgcgatccgtgctcaggaagatcgttcctcacagatcgaccacaacactgttgcttaccacttcaacgagccaatcggtgttgttggtcagatcattccttggaacttcccaatcctcatggctacctggaagctcgcaccggcacttgctgcaggtaacgcgatcgtcatgaagccagctgagcagaccccagcatccattttgtatctgattaacatcatcggcgatctcatcccagagggcgtcctcaacatcgtcaacggactcggcggtgaagcaggcgctgcactgtccggctctaatcggattggcaagattgctttcaccggttccaccgaggtcggcaagctgatcaaccgcgctgcatccgacaagatcattcctgtcaccctggagctcggcggtaagtccccatccatcttcttctccgatgttctgtcacaggatgacgccttcgcagagaaggcagttgaaggcttcgcgatgttcgccctcaatcagggtgaagtttgtacctgtccttcccgtgcacttgttcatgagtccatcgctgatgaattcctcgagcttggcgtgaagcgagttcagaacatcaagctgggtaacccacttgatactgaaaccatgatgggtgctcaggcgtcccaggagcagatggacaagatctcctcctacctgaagatcggcccagaagaaggcgctcaaaccctcactggtggcaaggtcaacaaggttgatggcatggagaacggttactacattgagccaaccgttttccgcggcaccaacgacatgaggatcttccgcgaggaaatcttcggaccagtcctttctgttgctaccttcagcgacttcgatgaggccatccgtattgcaaacgacaccaactacggcctcggcgctggtgtctggagccgtgaccaaaacaccatttatcgtgcaggtcgcgcaatccaggctggtcgagtttgggtcaaccagtaccacaactacccagcgcactccgctttcggtggatacaaggagtccggcatcggccgtgagaaccacctcatgatgctgaaccactaccagcagaccaagaacctgttggtctcctacgatccaaacccaaccggactgttctaa

SEQ ID NO: 12 - protein, 506 aa, Corynebacterium glutamicum
MTVYANPGTEGSIVNYEKRYENYIGGKWVPPVEGQYLENISPVTGEVFCEVARGTAADVELALDAAHAAADAWGKTSVAERALILHRIADRMEEHLEEIAVAETWENGKAVRETLAADIPLAIDHFRYFAGAIRAQEDRSSQIDHNTVAYHFNEPIGVVGQIIPWNFPILMATWKLAPALAAGNAIVMKPAEQTPASILYLINIIGDLIPEGVLNIVNGLGGEAGAALSGSNRIGKIAFTGSTEVGKLINRAASDKIIPVTLELGGKSPSIFFSDVLSQDDAFAEKAVEGFAMFALNQGEVCTCPSRALVHESIADEFLELGVKRVQNIKLGNPLDTETMMGAQASQEQMDKISSYLKIGPEEGAQTLTGGKVNKVDGMENGYYIEPTVFRGTNDMRIFREEIFGPVLSVATFSDFDEAIRIANDTNYGLGAGVWSRDQNTIYRAGRAIQAGRVWVNQYHNYPAHSAFGGYKESGIGRENHLMMLNHYQQTKNLLVSYDPNPTGLF

SEQ ID NO: 13 - DNA, 1356 bp, Carnobacterium divergens
  source 1..1356: mol_type = genomic DNA
atgaaagtagtagtagtaggctgtacacatgcaggaacagcggcagttaagacgattttaaatgaacatccagatgcatcagtatcagtatatgagcgtaatgacaatgtctcatttctatcttgtgggattgcgttgtatgttggtggagttgtgaaagatcctgcaggtttgttttattcaagtccagaagaacttgcatcaatgggcgcgaaaattaacatggaacacaatgtgaaaaatatagataatgagaataaggtcgtagtaattgagaatttaaaaacaggcgaaacatttgaagaaagctatgataagttggtaatgacaactggatcatggccaattattcctccaattgatggaatcaatagtgaaaatattcttttgtgtaaaaactataaccaagcaaatgaaattattaaagaatcaaaaaatgctaaaaagattgtcattgttggtggtggctatattggaattgaattagttgaggcatttgcagaatctggcaagcaagtgacgctagttgatggattagatcgtattttaaacaaatatttagatgctgaattcacttctgttttagagcatgatttacaagaaagaggcgttacgctagctttaaaccaaaccgtcgagaaatttgttgccaatgaatcaggtgctgtgacagctgtgaaaacaccagttggagaatatgaggctgatttagttattttatgtgttggatttaaaccaaatactgatttgttgaaggataaagtagagatgttgccaaatggtgccatcgtagtggatgaatatatgagaacaagcgatgaagcgatttttgctgctggcgatagttgcgcggttcattataatccaactggaggctctgcgtatattccgttagctacaaatgcagttagaatgggagctttagttgggaaaaatattgtttctccaacagttaaatatcgtggcacgcaagcaacttctggtttatatttatttggttttaatataggttcaaccggattgactgaaaatagcgctcctcattttggcgtagaggttcgttcagtagttgtagaagataattatcgtccagagtttatgccgacaacagagaaagtaacgatgaaattagtttatgaagtaggaacgaatcggattgttggaggtcaaatcatgtcaaaatatgatgtgacacaatctgccaatacgttatctttatgtgttcaaaataaaatgacgattgaggatttggcttatgtagatttcttcttccaacctcactttgatcgtccttggaactatttaaatattttagcgcaagcagctgttgagcaagagcgtaaactagcaaaataa

SEQ ID NO: 14 - protein, 451 aa, Carnobacterium divergens
MKVVVVGCTHAGTAAVKTILNEHPDASVSVYERNDNVSFLSCGIALYVGGVVKDPAGLFYSSPEELASMGAKINMEHNVKNIDNENKVVVIENLKTGETFEESYDKLVMTTGSWPIIPPIDGINSENILLCKNYNQANEIIKESKNAKKIVIVGGGYIGIELVEAFAESGKQVTLVDGLDRILNKYLDAEFTSVLEHDLQERGVTLALNQTVEKFVANESGAVTAVKTPVGEYEADLVILCVGFKPNTDLLKDKVEMLPNGAIVVDEYMRTSDEAIFAAGDSCAVHYNPTGGSAYIPLATNAVRMGALVGKNIVSPTVKYRGTQATSGLYLFGFNIGSTGLTENSAPHFGVEVRSVVVEDNYRPEFMPTTEKVTMKLVYEVGTNRIVGGQIMSKYDVTQSANTLSLCVQNKMTIEDLAYVDFFFQPHFDRPWNYLNILAQAAVEQERKLAK

SEQ ID NO: 15 - DNA, 1359 bp, Aerococcus urinaehominis
  source 1..1359: mol_type = genomic DNA
atgaaagttgcagtaatcggttgtacccatgctgggacagctgccgttaaaactatcttaacagaaaacgatgatgtagaagttgttgtttttgaacgcaatgataatatctccttcttatcttgtgggattgccctttacgtaggtggcgtggtcaaagacgtcaatggccttttctattctgatccaagtgagttagaatctctaggcgcaacagtttatatgaaacacaatgtgctatcgtttgacgaaaacactaaagttatccaagtagaaaatatggagactggcgaacatttccaagaatcatatgacaagttagtcattgccactggttcttggccgattattcctgatttaccaggactagatctagaaaatgtcatgctatgtaaaaactttaaacatgcccaagaattaatccaaactaagcaagataaaaaacgagttgctgttattggtgctggttatattggtatcgagttagttgaagcctttgctgaagacggtaaagaagttgttttaatcgatggtgctgaccgcgtcctacctaagtatctcgaccaggaaatgactgacttattagaagctagcttggtagaccatggcgtacaaatgcaattaggggaatttgtagaatcattcctagccgacgatgaaggtaaggtacgtgccgttaaaacgtctaaaggtgaatatgaatgtgatatggcagtcctttgtgtcggcttccaacctaacacagaattatataagggcaagttagaaactatgccgaatggtgcgattattgtagatgactatatgcacacctctcacccagatatctatgcctgtggtgactcatgtgctgtcaactataatcctaacgatggccatgcttatatcccgcttgccactaatgctgtccgtatgggtagcttagttggtaaaaatattaaagcagaccgcgtcaaataccggggcacccagtcaacatctggtctaaaattattcggctggaatattggctcaactggtgttaccgacaattctgctagcagcttcaaccttgaaactcgtagcgtctatgttgaagataactaccgccctgaattcatgcctactacagaaaaagtttatatgaagttagtctatgaagtaggcacaaatcgagttgttggcggtcagcttatgtctaagtatgatattacccaatcagccaacaccctatcactagctatccaaaccaagcaaacaattgaagatttagcctatgtggacttcttcttccaaccacactttgaccgcccttggaactatttaaatattttagcccaagcagcactaagtcaagaagaagaattagctcaaaactaa

SEQ ID NO: 16 - protein, 452 aa, Aerococcus urinaehominis
MKVAVIGCTHAGTAAVKTILTENDDVEVVVFERNDNISFLSCGIALYVGGVVKDVNGLFYSDPSELESLGATVYMKHNVLSFDENTKVIQVENMETGEHFQESYDKLVIATGSWPIIPDLPGLDLENVMLCKNFKHAQELIQTKQDKKRVAVIGAGYIGIELVEAFAEDGKEVVLIDGADRVLPKYLDQEMTDLLEASLVDHGVQMQLGEFVESFLADDEGKVRAVKTSKGEYECDMAVLCVGFQPNTELYKGKLETMPNGAIIVDDYMHTSHPDIYACGDSCAVNYNPNDGHAYIPLATNAVRMGSLVGKNIKADRVKYRGTQSTSGLKLFGWNIGSTGVTDNSASSFNLETRSVYVEDNYRPEFMPTTEKVYMKLVYEVGTNRVVGGQLMSKYDITQSANTLSLAIQTKQTIEDLAYVDFFFQPHFDRPWNYLNILAQAALSQEEELAQN

SEQ ID NO: 17 - DNA, 1374 bp, Desemzia incerta
  source 1..1374: mol_type = genomic DNA
atgaaagtagtcgttgtaggatgtacgcacgctggaacatcagcagtaaaaacaattcttaatgagcatccaaatactgaagtaacagtttttgaacgaaatgataatgtgtcattcttatcatgcggaatcgcattgtatgttggtggcgttgtgaaagatccagcaggtttattctattcaaatcctgaagaattaactgaaatgggcgcaactgtgcacatggaacacaatgttacaaatatcgatactgttgctaaaaaagttactgtagaaaatatgcaaactggtgaagtctttgaagaatcatacgacaaattagtgaatacaacaggttcatggccgattgttccaccaatctctggtattgagtctaaaaacattttattatgtaaaaactacaaccaagctaatgaaatcattcgccaagcaaaagacaaacaaaaagttgttattgttggtggaggttacattggtattgaattagtggaagcgtttgctgaatctggaaaagatgttacgttgattgatggattagaccgtattttaaacaaatacctagatccagaattcacagatatcttagaacacgatttgcaagaacgtggaatcaaattagcactaaaccaaactgtaaatggctttgaagcgaatgaaaatggagaagtaactaaagttgtcacttctgaaaattcatttgaaactgaaatggttatcatgtgtgttggtttccgtccaaacaatgaattgttaaaagacaaagtagatatgttgccaaatggcgctattattgttgatgaatacatgagaacaagcgataaagatatttacgctgctggagacagctgtgcagttcattacaatccaaatggtggatctgcatatattccattagcaactaacgctgttcgcatgggaactttagttggtaaaaacattgttgaaccaagtgttaaataccgtggaacacaatctacatctggattgtacttgttcggtttcaacatcggttctacaggagtaaacgtaaacagtgcttctcatttcggattagatgttcgttcagttgtagttgaagactactaccgtccagaattcatgccgacaaatgaaaaagtattgatgaaattagtttatgaagttggaacaaaccgcatcgttggtggacaagtaatgtctaaatatgacatcactcaatcagctaatacattgtcattagctgtacaaaacaaaatgactatcgaagatttggcatatgttgacttcttcttccaaccagtattcgatcgtccttggaactacttgaacttgcttgcacaagcagcagtagaacaagaaagaaaaatcgcaacaggtacagaagtaactgtttaa

SEQ ID NO: 18 - protein, 457 aa, Desemzia incerta
MKVVVVGCTHAGTSAVKTILNEHPNTEVTVFERNDNVSFLSCGIALYVGGVVKDPAGLFYSNPEELTEMGATVHMEHNVTNIDTVAKKVTVENMQTGEVFEESYDKLVNTTGSWPIVPPISGIESKNILLCKNYNQANEIIRQAKDKQKVVIVGGGYIGIELVEAFAESGKDVTLIDGLDRILNKYLDPEFTDILEHDLQERGIKLALNQTVNGFEANENGEVTKVVTSENSFETEMVIMCVGFRPNNELLKDKVDMLPNGAIIVDEYMRTSDKDIYAAGDSCAVHYNPNGGSAYIPLATNAVRMGTLVGKNIVEPSVKYRGTQSTSGLYLFGFNIGSTGVNVNSASHFGLDVRSVVVEDYYRPEFMPTNEKVLMKLVYEVGTNRIVGGQVMSKYDITQSANTLSLAVQNKMTIEDLAYVDFFFQPVFDRPWNYLNLLAQAAVEQERKIATGTEVTV